European Patent Application EP 4 148 132 A1, published March 15, 2023. Title: NOVEL NUCLEIC ACID LIGANDS AND METHOD FOR IDENTIFYING THEREOF. Applicant: INTEROLIGO Corporation. The sequence listing filed with the application follows.

SEQUENCE LISTING (185 sequences)

SEQ ID NO: 1 - DNA, 74 bp, Artificial Sequence
  DNA library template
  N_region (17)..(57): a, g, c, or t
gctggtggtgtggctgnnnnnnnnnnnnnnnnnnnnnnnnnnnnnnnnnnnnnnnncaggcagacggtcactca

SEQ ID NO: 2 - DNA, 17 bp, Artificial Sequence
  5' primer
gagtgaccgtctgcctg

SEQ ID NO: 3 - DNA, 16 bp, Artificial Sequence
  biotin-3' primer
gctggtggtgtggctg

SEQ ID NO: 4 - DNA, 17 bp, Artificial Sequence
  biotin-5' primer
gagtgaccgtctgcctg

SEQ ID NO: 5 - DNA, 16 bp, Artificial Sequence
  3' primer
gctggtggtgtggctg

SEQ ID NO: 6 - DNA, 74 bp, Artificial Sequence
  nucleic acid ligand AA001, wherein n is 5-(N-(1-naphthylmethyl)carboxamide)-2'-deoxyuridine(Nap-dU)
gagtgaccgtctgccngganccngcccnnnnaanccgacnnnaanggccacgcncaccagccacaccaccagcc

SEQ ID NO: 7 - DNA, 50 bp, Artificial Sequence
  nucleic acid ligand AA002, wherein n is 5-(N-(1-naphthylmethyl)carboxamide)-2'-deoxyuridine(Nap-dU)
gcctgganccngcccnnnnaanccgacnnnaanggccacgcncaccagcc

SEQ ID NO: 8 - DNA, 40 bp, Artificial Sequence
  nucleic acid ligand AA003, wherein n is 5-(N-(1-naphthylmethyl)carboxamide)-2'-deoxyuridine(Nap-dU)
ganccngcccnnnnaanccgacnnnaanggccacgcncac

SEQ ID NO: 9 - DNA, 35 bp, Artificial Sequence
  nucleic acid ligand AA004, wherein n is 5-(N-(1-naphthylmethyl)carboxamide)-2'-deoxyuridine(Nap-dU)
ngcccnnnnaanccgacnnnaanggccacgcncac

SEQ ID NO: 10 - DNA, 30 bp, Artificial Sequence
  nucleic acid ligand AA005, wherein n is 5-(N-(1-naphthylmethyl)carboxamide)-2'-deoxyuridine(Nap-dU)
ngcccnnnnaanccgacnnnaanggccacg

SEQ ID NO: 11 - DNA, 26 bp, Artificial Sequence
  nucleic acid ligand AA006, wherein n is 5-(N-(1-naphthylmethyl)carboxamide)-2'-deoxyuridine(Nap-dU)
ngcccnnnnaanccgacnnnaanggc

SEQ ID NO: 12 - DNA, 22 bp, Artificial Sequence
  nucleic acid ligand AA007, wherein n is 5-(N-(1-naphthylmethyl)carboxamide)-2'-deoxyuridine(Nap-dU)
gcccnnnnaanccgacnnnaan

SEQ ID NO: 13 - DNA, 75 bp, Artificial Sequence
  nucleic acid ligand AB001, wherein n is 5-(N-(1-naphthylmethyl)carboxamide)-2'-deoxyuridine(Nap-dU)
gagtgaccgtctgccngncnccaaccncgccnnnacaacnanancngacgaacnaacacagccacaccaccagcc

SEQ ID NO: 14 - DNA, 51 bp, Artificial Sequence
  nucleic acid ligand AB002, wherein n is 5-(N-(1-naphthylmethyl)carboxamide)-2'-deoxyuridine(Nap-dU)
gcctgncnccaaccncgccnnnacaacnanancngacgaacnaacacagcc

SEQ ID NO: 15 - DNA, 41 bp, Artificial Sequence
  nucleic acid ligand AB003, wherein n is 5-(N-(1-naphthylmethyl)carboxamide)-2'-deoxyuridine(Nap-dU)
ncnccaaccncgccnnnacaacnanancngacgaacnaaca

SEQ ID NO: 16 - DNA, 36 bp, Artificial Sequence
  nucleic acid ligand AB004, wherein n is 5-(N-(1-naphthylmethyl)carboxamide)-2'-deoxyuridine(Nap-dU)
aaccncgccnnnacaacnanancngacgaacnaaca

SEQ ID NO: 17 - DNA, 31 bp, Artificial Sequence
  nucleic acid ligand AB005, wherein n is 5-(N-(1-naphthylmethyl)carboxamide)-2'-deoxyuridine(Nap-dU)
aaccncgccnnnacaacnanancngacgaac

SEQ ID NO: 18 - DNA, 27 bp, Artificial Sequence
  nucleic acid ligand AB006, wherein n is 5-(N-(1-naphthylmethyl)carboxamide)-2'-deoxyuridine(Nap-dU)
ncgccnnnacaacnanancngacgaac

SEQ ID NO: 19 - DNA, 25 bp, Artificial Sequence
  nucleic acid ligand AB007, wherein n is 5-(N-(1-naphthylmethyl)carboxamide)-2'-deoxyuridine(Nap-dU)
ncgccnnnacaacnanancngacga

SEQ ID NO: 20 - DNA, 78 bp, Artificial Sequence
  nucleic acid ligand AD001, wherein n is 5-(N-(1-naphthylmethyl)carboxamide)-2'-deoxyuridine(Nap-dU)
gagtgaccgtctgcctgngngagaannangnaccnnaacgancanccgaaggnnnngaccacagccacaccaccagcc

SEQ ID NO: 21 - DNA, 78 bp, Artificial Sequence
  nucleic acid ligand AD002, wherein n is 5-(N-(1-naphthylmethyl)carboxamide)-2'-deoxyuridine(Nap-dU)
gagtgaccgtctgcctgngncngagggacccnnnnnaagggcannancagcangccncacacagccacaccaccagcc

SEQ ID NO: 22 - DNA, 73 bp, Artificial Sequence
  nucleic acid ligand AD003, wherein n is 5-(N-(1-naphthylmethyl)carboxamide)-2'-deoxyuridine(Nap-dU)
gagtgaccgtcngcctggacnagcanaagnccgganggcagcnnnangccgaccancagccacaccaccagcc

SEQ ID NO: 23 - DNA, 49 bp, Artificial Sequence
  nucleic acid ligand AD004, wherein n is 5-(N-(1-naphthylmethyl)carboxamide)-2'-deoxyuridine(Nap-dU)
gcctggacnagcanaagnccgganggcagcnnnangccgaccancagcc

SEQ ID NO: 24 - DNA, 39 bp, Artificial Sequence
  nucleic acid ligand AD005, wherein n is 5-(N-(1-naphthylmethyl)carboxamide)-2'-deoxyuridine(Nap-dU)
gacnagcanaagnccgganggcagcnnnangccgaccan

SEQ ID NO: 25 - DNA, 34 bp, Artificial Sequence
  nucleic acid ligand AD006, wherein n is 5-(N-(1-naphthylmethyl)carboxamide)-2'-deoxyuridine(Nap-dU)
gacnagcanaagnccgganggcagcnnnangccg

SEQ ID NO: 26 - DNA, 32 bp, Artificial Sequence
  nucleic acid ligand AD007, wherein n is 5-(N-(1-naphthylmethyl)carboxamide)-2'-deoxyuridine(Nap-dU)
gcanaagnccgganggcagcnnnangccgacc

SEQ ID NO: 27 - DNA, 27 bp, Artificial Sequence
  nucleic acid ligand AD008, wherein n is 5-(N-(1-naphthylmethyl)carboxamide)-2'-deoxyuridine(Nap-dU)
gcanaagnccgganggcagcnnnangc

SEQ ID NO: 28 - DNA, 74 bp, Artificial Sequence
  nucleic acid ligand AD009, wherein n is 5-(N-(1-naphthylmethyl)carboxamide)-2'-deoxyuridine(Nap-dU)
gagtgaccgtctgccngccccgccncnncngaagnnaacangngcnccgaganggnacagccacaccaccagcc

SEQ ID NO: 29 - DNA, 50 bp, Artificial Sequence
  nucleic acid ligand AD010, wherein n is 5-(N-(1-naphthylmethyl)carboxamide)-2'-deoxyuridine(Nap-dU)
gcctgccccgccncnncngaagnnaacangngcnccgaganggnacagcc

SEQ ID NO: 30 - DNA, 40 bp, Artificial Sequence
  nucleic acid ligand AD011, wherein n is 5-(N-(1-naphthylmethyl)carboxamide)-2'-deoxyuridine(Nap-dU)
ccccgccncnncngaagnnaacangngcnccgaganggna

SEQ ID NO: 31 - DNA, 35 bp, Artificial Sequence
  nucleic acid ligand AD012, wherein n is 5-(N-(1-naphthylmethyl)carboxamide)-2'-deoxyuridine(Nap-dU)
ccccgccncnncngaagnnaacangngcnccgaga

SEQ ID NO: 32 - DNA, 30 bp, Artificial Sequence
  nucleic acid ligand AD013, wherein n is 5-(N-(1-naphthylmethyl)carboxamide)-2'-deoxyuridine(Nap-dU)
ccncnncngaagnnaacangngcnccgaga

SEQ ID NO: 33 - DNA, 31 bp, Artificial Sequence
  nucleic acid ligand AD014, wherein n is 5-(N-(1-naphthylmethyl)carboxamide)-2'-deoxyuridine(Nap-dU)
ccccgccncnncngaagnnaacangngcncc

SEQ ID NO: 34 - DNA, 26 bp, Artificial Sequence
  nucleic acid ligand AD015, wherein n is 5-(N-(1-naphthylmethyl)carboxamide)-2'-deoxyuridine(Nap-dU)
ccncnncngaagnnaacangngcncc

SEQ ID NO: 35 - DNA, 29 bp, Artificial Sequence
  nucleic acid ligand AD016, wherein n is 5-(N-(1-naphthylmethyl)carboxamide)-2'-deoxyuridine(Nap-dU)
gacnagcanaagnccgganggcagcnnna

SEQ ID NO: 36 - DNA, 24 bp, Artificial Sequence
  nucleic acid ligand AD017, wherein n is 5-(N-(1-naphthylmethyl)carboxamide)-2'-deoxyuridine(Nap-dU)
gacnagcanaagnccgganggcag

SEQ ID NO: 37 - DNA, 19 bp, Artificial Sequence
  nucleic acid ligand AD018, wherein n is 5-(N-(1-naphthylmethyl)carboxamide)-2'-deoxyuridine(Nap-dU)
gacnagcanaagnccggan

SEQ ID NO: 38 - DNA, 29 bp, Artificial Sequence
  nucleic acid ligand AD020, wherein n is 5-(N-(1-naphthylmethyl)carboxamide)-2'-deoxyuridine(Nap-dU)
agnccgganggcagcnnnangccgaccan

SEQ ID NO: 39 - DNA, 26 bp, Artificial Sequence
  nucleic acid ligand AD024, wherein n is 5-(N-(1-naphthylmethyl)carboxamide)-2'-deoxyuridine(Nap-dU)
gcanaagnccgganggcagcnnnang

SEQ ID NO: 40 - DNA, 22 bp, Artificial Sequence
  nucleic acid ligand AD025, wherein n is 5-(N-(1-naphthylmethyl)carboxamide)-2'-deoxyuridine(Nap-dU)
agnccgganggcagcnnnangc

SEQ ID NO: 41 - DNA, 29 bp, Artificial Sequence
  nucleic acid ligand AD026, wherein n is 5-(N-(1-naphthylmethyl)carboxamide)-2'-deoxyuridine(Nap-dU)
nagcanaagnccgganggcagcnnnangc

SEQ ID NO: 42 - DNA, 57 bp, Artificial Sequence
  nucleic acid ligand AD032, wherein n is 5-(N-(1-naphthylmethyl)carboxamide)-2'-deoxyuridine(Nap-dU)
caggncgagcngnacgcgngngngaccngaagacgnanaacnnnnacagaancnaca

SEQ ID NO: 43 - DNA, 57 bp, Artificial Sequence
  nucleic acid ligand AD034, wherein n is 5-(N-(1-naphthylmethyl)carboxamide)-2'-deoxyuridine(Nap-dU)
caggncgagcngnacgcgngngngaccngccccacnncngacannagacngngnaga

SEQ ID NO: 44 - DNA, 53 bp, Artificial Sequence
  nucleic acid ligand AD036, wherein n is 5-(N-(1-naphthylmethyl)carboxamide)-2'-deoxyuridine(Nap-dU)
caggncgagcngnacgcgngngngaccngccccacnncngacannagacngng

SEQ ID NO: 45 - DNA, 52 bp, Artificial Sequence
  nucleic acid ligand AD037, wherein n is 5-(N-(1-naphthylmethyl)carboxamide)-2'-deoxyuridine(Nap-dU)
caggncgagcngnacgcgngngngaccngccccacnncngacannagacngn

SEQ ID NO: 46 - DNA, 51 bp, Artificial Sequence
  nucleic acid ligand AD038, wherein n is 5-(N-(1-naphthylmethyl)carboxamide)-2'-deoxyuridine(Nap-dU)
caggncgagcngnacgcgngngngaccngccccacnncngacannagacng

SEQ ID NO: 47 - DNA, 48 bp, Artificial Sequence
  nucleic acid ligand AD039, wherein n is 5-(N-(1-naphthylmethyl)carboxamide)-2'-deoxyuridine(Nap-dU)
caggncgagcngnacgcgngngngaccngccccacnncngacannaga

SEQ ID NO: 48 - DNA, 47 bp, Artificial Sequence
  nucleic acid ligand AD040, wherein n is 5-(N-(1-naphthylmethyl)carboxamide)-2'-deoxyuridine(Nap-dU)
caggncgagcngnacgcgngngngaccngccccacnncngacannag

SEQ ID NO: 49 - DNA, 35 bp, Artificial Sequence
  nucleic acid ligand AD041, wherein n is 5-(N-(1-naphthylmethyl)carboxamide)-2'-deoxyuridine(Nap-dU)
nacgcgngngngaccngccccacnncngacannag

SEQ ID NO: 50 - DNA, 38 bp, Artificial Sequence
  nucleic acid ligand AD059, wherein n is 5-(N-(1-naphthylmethyl)carboxamide)-2'-deoxyuridine(Nap-dU)
gacnagcanaagnccgganggcagcnnnangccgacca

SEQ ID NO: 51 - DNA, 37 bp, Artificial Sequence
  nucleic acid ligand AD060, wherein n is 5-(N-(1-naphthylmethyl)carboxamide)-2'-deoxyuridine(Nap-dU)
gacnagcanaagnccgganggcagcnnnangccgacc

SEQ ID NO: 52 - DNA, 33 bp, Artificial Sequence
  nucleic acid ligand AD061, wherein n is 5-(N-(1-naphthylmethyl)carboxamide)-2'-deoxyuridine(Nap-dU)
gacnagcanaagnccgganggcagcnnnangcc

SEQ ID NO: 53 - DNA, 31 bp, Artificial Sequence
  nucleic acid ligand AD063, wherein n is 5-(N-(1-naphthylmethyl)carboxamide)-2'-deoxyuridine(Nap-dU)
gacnagcanaagnccgganggcagcnnnang

SEQ ID NO: 54 - DNA, 30 bp, Artificial Sequence
  nucleic acid ligand AD064, wherein n is 5-(N-(1-naphthylmethyl)carboxamide)-2'-deoxyuridine(Nap-dU)
gacnagcanaagnccgganggcagcnnnan

SEQ ID NO: 55 - DNA, 25 bp, Artificial Sequence
  nucleic acid ligand AD065, wherein n is 5-(N-(1-naphthylmethyl)carboxamide)-2'-deoxyuridine(Nap-dU)
gacnagcanaagnccgganggcagc

SEQ ID NO: 56 - DNA, 25 bp, Artificial Sequence
  nucleic acid ligand AD066, wherein n is 5-(N-(1-naphthylmethyl)carboxamide)-2'-deoxyuridine(Nap-dU)
canaagnccgganggcagcnnnang

SEQ ID NO: 57 - DNA, 23 bp, Artificial Sequence
  nucleic acid ligand AD067, wherein n is 5-(N-(1-naphthylmethyl)carboxamide)-2'-deoxyuridine(Nap-dU)
anaagnccgganggcagcnnnan

SEQ ID NO: 58 - DNA, 19 bp, Artificial Sequence
  nucleic acid ligand AD068, wherein n is 5-(N-(1-naphthylmethyl)carboxamide)-2'-deoxyuridine(Nap-dU)
aagnccgganggcagcnnn

SEQ ID NO: 59 - DNA, 18 bp, Artificial Sequence
  nucleic acid ligand AD069, wherein n is 5-(N-(1-naphthylmethyl)carboxamide)-2'-deoxyuridine(Nap-dU)
agnccgganggcagcnnn

SEQ ID NO: 60 - DNA, 18 bp, Artificial Sequence
  nucleic acid ligand AD070, wherein n is 5-(N-(1-naphthylmethyl)carboxamide)-2'-deoxyuridine(Nap-dU)
aagnccgganggcagcnn

SEQ ID NO: 61 - DNA, 15 bp, Artificial Sequence
  nucleic acid ligand AD071, wherein n is 5-(N-(1-naphthylmethyl)carboxamide)-2'-deoxyuridine(Nap-dU)
gacnagcanaagncc

SEQ ID NO: 62 - DNA, 14 bp, Artificial Sequence
  nucleic acid ligand AD072, wherein n is 5-(N-(1-naphthylmethyl)carboxamide)-2'-deoxyuridine(Nap-dU)
gacnagcanaagnc

SEQ ID NO: 63 - DNA, 13 bp, Artificial Sequence
  nucleic acid ligand AD073, wherein n is 5-(N-(1-naphthylmethyl)carboxamide)-2'-deoxyuridine(Nap-dU)
gacnagcanaagn

SEQ ID NO: 64 - DNA, 17 bp, Artificial Sequence
  nucleic acid ligand AD078, wherein n is 5-(N-(1-naphthylmethyl)carboxamide)-2'-deoxyuridine(Nap-dU)
agcnnnangccgaccan

SEQ ID NO: 65 - DNA, 16 bp, Artificial Sequence
  nucleic acid ligand AD079, wherein n is 5-(N-(1-naphthylmethyl)carboxamide)-2'-deoxyuridine(Nap-dU)
gcnnnangccgaccan

SEQ ID NO: 66 - DNA, 33 bp, Artificial Sequence
  nucleic acid ligand AD080, wherein n is 5-(N-(1-naphthylmethyl)carboxamide)-2'-deoxyuridine(Nap-dU)
ncnncngaagnnaacangngcnccgaganggna

SEQ ID NO: 67 - DNA, 32 bp, Artificial Sequence
  nucleic acid ligand AD081, wherein n is 5-(N-(1-naphthylmethyl)carboxamide)-2'-deoxyuridine(Nap-dU)
ncnncngaagnnaacangngcnccgaganggn

SEQ ID NO: 68 - DNA, 32 bp, Artificial Sequence
  nucleic acid ligand AD083, wherein n is 5-(N-(1-naphthylmethyl)carboxamide)-2'-deoxyuridine(Nap-dU)
cnncngaagnnaacangngcnccgaganggna

SEQ ID NO: 69 - DNA, 12 bp, Artificial Sequence
  nucleic acid ligand AD084, wherein n is 5-(N-(1-naphthylmethyl)carboxamide)-2'-deoxyuridine(Nap-dU)
nccgaganggna

SEQ ID NO: 70 - DNA, 39 bp, Artificial Sequence
  nucleic acid ligand AD085, wherein n is 5-(N-(1-naphthylmethyl)carboxamide)-2'-deoxyuridine(Nap-dU)
ccccgccncnncngaagnnaacangngcnccgaganggn

SEQ ID NO: 71 - DNA, 38 bp, Artificial Sequence
  nucleic acid ligand AD086, wherein n is 5-(N-(1-naphthylmethyl)carboxamide)-2'-deoxyuridine(Nap-dU)
ccccgccncnncngaagnnaacangngcnccgagangg

SEQ ID NO: 72 - DNA, 50 bp, Artificial Sequence
  nucleic acid ligand AP001, wherein n is 5-(N-(1-naphthylmethyl)carboxamide)-2'-deoxyuridine(Nap-dU)
gccngacaacaacgagngcgaacngnacnacnnganagagacccncagcc

SEQ ID NO: 73 - DNA, 40 bp, Artificial Sequence
  nucleic acid ligand AP002, wherein n is 5-(N-(1-naphthylmethyl)carboxamide)-2'-deoxyuridine(Nap-dU)
acaacaacgagngcgaacngnacnacnnganagagacccn

SEQ ID NO: 74 - DNA, 36 bp, Artificial Sequence
  nucleic acid ligand AP003, wherein n is 5-(N-(1-naphthylmethyl)carboxamide)-2'-deoxyuridine(Nap-dU)
caacgagngcgaacngnacnacnnganagagacccn

SEQ ID NO: 75 - DNA, 32 bp, Artificial Sequence
  nucleic acid ligand AP004, wherein n is 5-(N-(1-naphthylmethyl)carboxamide)-2'-deoxyuridine(Nap-dU)
caacgagngcgaacngnacnacnnganagaga

SEQ ID NO: 76 - DNA, 29 bp, Artificial Sequence
  nucleic acid ligand AP005, wherein n is 5-(N-(1-naphthylmethyl)carboxamide)-2'-deoxyuridine(Nap-dU)
cgagngcgaacngnacnacnnganagaga

SEQ ID NO: 77 - DNA, 26 bp, Artificial Sequence
  nucleic acid ligand AP006, wherein n is 5-(N-(1-naphthylmethyl)carboxamide)-2'-deoxyuridine(Nap-dU)
cgagngcgaacngnacnacnnganag

SEQ ID NO: 78 - DNA, 50 bp, Artificial Sequence
  nucleic acid ligand AP007, wherein n is 5-(N-(1-naphthylmethyl)carboxamide)-2'-deoxyuridine(Nap-dU)
gccnggagcanggncacangnacnacnnganaggagcccgngccncagcc

SEQ ID NO: 79 - DNA, 40 bp, Artificial Sequence
  nucleic acid ligand AP008, wherein n is 5-(N-(1-naphthylmethyl)carboxamide)-2'-deoxyuridine(Nap-dU)
gagcanggncacangnacnacnnganaggagcccgngccn

SEQ ID NO: 80 - DNA, 37 bp, Artificial Sequence
  nucleic acid ligand AP009, wherein n is 5-(N-(1-naphthylmethyl)carboxamide)-2'-deoxyuridine(Nap-dU)
canggncacangnacnacnnganaggagcccgngccn

SEQ ID NO: 81 - DNA, 32 bp, Artificial Sequence
  nucleic acid ligand AP010, wherein n is 5-(N-(1-naphthylmethyl)carboxamide)-2'-deoxyuridine(Nap-dU)
canggncacangnacnacnnganaggagcccg

SEQ ID NO: 82 - DNA, 29 bp, Artificial Sequence
  nucleic acid ligand AP011, wherein n is 5-(N-(1-naphthylmethyl)carboxamide)-2'-deoxyuridine(Nap-dU)
canggncacangnacnacnnganaggagc

SEQ ID NO: 83 - DNA, 25 bp, Artificial Sequence
  nucleic acid ligand AP012, wherein n is 5-(N-(1-naphthylmethyl)carboxamide)-2'-deoxyuridine(Nap-dU)
canggncacangnacnacnnganag

SEQ ID NO: 84 - DNA, 74 bp, Artificial Sequence
  nucleic acid ligand AP013, wherein n is 5-(N-(1-naphthylmethyl)carboxamide)-2'-deoxyuridine(Nap-dU)
gagtgaccgtctgcctgacaacaacgagngcgaacngnacnacnnganagagacccncagccacaccaccagcc

SEQ ID NO: 85 - DNA, 74 bp, Artificial Sequence
  nucleic acid ligand AP014, wherein n is 5-(N-(1-naphthylmethyl)carboxamide)-2'-deoxyuridine(Nap-dU)
gagtgaccgtctgcctggagcanggncacangnacnacnnganaggagcccgngccncagccacaccaccagcc

SEQ ID NO: 86 - DNA, 50 bp, Artificial Sequence
  nucleic acid ligand AP015, wherein n is 5-(N-(1-naphthylmethyl)carboxamide)-2'-deoxyuridine(Nap-dU)
gcctgncaancacngacgaaangnacnacnnganagagcnaaccncagcc

SEQ ID NO: 87 - DNA, 40 bp, Artificial Sequence
  nucleic acid ligand AP016, wherein n is 5-(N-(1-naphthylmethyl)carboxamide)-2'-deoxyuridine(Nap-dU)
ncaancacngacgaaangnacnacnnganagagcnaaccn

SEQ ID NO: 88 - DNA, 35 bp, Artificial Sequence
  nucleic acid ligand AP017, wherein n is 5-(N-(1-naphthylmethyl)carboxamide)-2'-deoxyuridine(Nap-dU)
cacngacgaaangnacnacnnganagagcnaaccn

SEQ ID NO: 89 - DNA, 30 bp, Artificial Sequence
  nucleic acid ligand AP018, wherein n is 5-(N-(1-naphthylmethyl)carboxamide)-2'-deoxyuridine(Nap-dU)
cacngacgaaangnacnacnnganagagcn

SEQ ID NO: 90 - DNA, 27 bp, Artificial Sequence
  nucleic acid ligand AP019, wherein n is 5-(N-(1-naphthylmethyl)carboxamide)-2'-deoxyuridine(Nap-dU)
ngacgaaangnacnacnnganagagcn

SEQ ID NO: 91 - DNA, 23 bp, Artificial Sequence
  nucleic acid ligand AP020, wherein n is 5-(N-(1-naphthylmethyl)carboxamide)-2'-deoxyuridine(Nap-dU)
acgaaangnacnacnnganagag

SEQ ID NO: 92 - DNA, 69 bp, Artificial Sequence
  nucleic acid ligand AP021, wherein n is 5-(N-(1-naphthylmethyl)carboxamide)-2'-deoxyuridine(Nap-dU)
accgtctgcctgacaacaacgagngcgaacngnacnacnnganagagacccncagccacaccaccagcc

SEQ ID NO: 93 - DNA, 66 bp, Artificial Sequence
  nucleic acid ligand AP022, wherein n is 5-(N-(1-naphthylmethyl)carboxamide)-2'-deoxyuridine(Nap-dU)
gtctgcctgacaacaacgagngcgaacngnacnacnnganagagacccncagccacaccaccagcc

SEQ ID NO: 94 - DNA, 58 bp, Artificial Sequence
  nucleic acid ligand AP023, wherein n is 5-(N-(1-naphthylmethyl)carboxamide)-2'-deoxyuridine(Nap-dU)
gagtgaccgtctgcctgacaacaacgagngcgaacngnacnacnnganagagacccnc

SEQ ID NO: 95 - DNA, 50 bp, Artificial Sequence
  nucleic acid ligand AP024, wherein n is 5-(N-(1-naphthylmethyl)carboxamide)-2'-deoxyuridine(Nap-dU)
gtctgcctgacaacaacgagngcgaacngnacnacnnganagagacccnc

SEQ ID NO: 96 - DNA, 49 bp, Artificial Sequence
  nucleic acid ligand AP025, wherein n is 5-(N-(1-naphthylmethyl)carboxamide)-2'-deoxyuridine(Nap-dU)
gtctgcctgacaacaacgagngcgaacngnacnacnnganagagacccn

SEQ ID NO: 97 - DNA, 44 bp, Artificial Sequence
  nucleic acid ligand AP026, wherein n is 5-(N-(1-naphthylmethyl)carboxamide)-2'-deoxyuridine(Nap-dU)
gtctgcctgacaacaacgagngcgaacngnacnacnnganagag

SEQ ID NO: 98 - DNA, 74 bp, Artificial Sequence
  nucleic acid ligand AP027, wherein n is 5-(N-(1-naphthylmethyl)carboxamide)-2'-deoxyuridine(Nap-dU)
gagtgaccgtctgcctgncaancacngacgaaangnacnacnnganagagcnaaccncagccacaccaccagcc

SEQ ID NO: 99 - DNA, 58 bp, Artificial Sequence
  nucleic acid ligand AP030, wherein n is 5-(N-(1-naphthylmethyl)carboxamide)-2'-deoxyuridine(Nap-dU)
ncccaggncgagcngnacgcgngngngaccacngnacnacnnganagaggcacngccn

SEQ ID NO: 100 - DNA, 58 bp, Artificial Sequence
  nucleic acid ligand AP031, wherein n is 5-(N-(1-naphthylmethyl)carboxamide)-2'-deoxyuridine(Nap-dU)
ncccaggncgagcngnacgcgngngngaccnnacnganaancaccnngaanagngnac

SEQ ID NO: 101 - DNA, 55 bp, Artificial Sequence
  nucleic acid ligand AP033, wherein n is 5-(N-(1-naphthylmethyl)carboxamide)-2'-deoxyuridine(Nap-dU)
caggncgagcngnacgcgngngngaccnnacnganaancaccnngaanagngnac

SEQ ID NO: 102 - DNA, 48 bp, Artificial Sequence
  nucleic acid ligand AP034, wherein n is 5-(N-(1-naphthylmethyl)carboxamide)-2'-deoxyuridine(Nap-dU)
agcngnacgcgngngngaccnnacnganaancaccnngaanagngnac

SEQ ID NO: 103 - DNA, 43 bp, Artificial Sequence
  nucleic acid ligand AP035, wherein n is 5-(N-(1-naphthylmethyl)carboxamide)-2'-deoxyuridine(Nap-dU)
nacgcgngngngaccnnacnganaancaccnngaanagngnac

SEQ ID NO: 104 - DNA, 38 bp, Artificial Sequence
  nucleic acid ligand AP036, wherein n is 5-(N-(1-naphthylmethyl)carboxamide)-2'-deoxyuridine(Nap-dU)
gngngngaccnnacnganaancaccnngaanagngnac

SEQ ID NO: 105 - DNA, 31 bp, Artificial Sequence
  nucleic acid ligand AP037, wherein n is 5-(N-(1-naphthylmethyl)carboxamide)-2'-deoxyuridine(Nap-dU)
accnnacnganaancaccnngaanagngnac

SEQ ID NO: 106 - DNA, 38 bp, Artificial Sequence
  nucleic acid ligand AP038, wherein n is 5-(N-(1-naphthylmethyl)carboxamide)-2'-deoxyuridine(Nap-dU)
ncccaggncgagcngnacgcgngngngaccnnacngan

SEQ ID NO: 107 - DNA, 43 bp, Artificial Sequence
  nucleic acid ligand AP039, wherein n is 5-(N-(1-naphthylmethyl)carboxamide)-2'-deoxyuridine(Nap-dU)
ncccaggncgagcngnacgcgngngngaccnnacnganaanca

SEQ ID NO: 108 - DNA, 52 bp, Artificial Sequence
  nucleic acid ligand AP040, wherein n is 5-(N-(1-naphthylmethyl)carboxamide)-2'-deoxyuridine(Nap-dU)
ncccaggncgagcngnacgcgngngngaccnnacnganaancaccnngaana

SEQ ID NO: 109 - DNA, 42 bp, Artificial Sequence
  nucleic acid ligand AP045, wherein n is 5-(N-(1-naphthylmethyl)carboxamide)-2'-deoxyuridine(Nap-dU)
canggncacangnacnacnnganaggagcccgngccncagcc

SEQ ID NO: 110 - DNA, 39 bp, Artificial Sequence
  nucleic acid ligand AP046, wherein n is 5-(N-(1-naphthylmethyl)carboxamide)-2'-deoxyuridine(Nap-dU)
ggncacangnacnacnnganaggagcccgngccncagcc

SEQ ID NO: 111 - DNA, 38 bp, Artificial Sequence
  nucleic acid ligand AP047, wherein n is 5-(N-(1-naphthylmethyl)carboxamide)-2'-deoxyuridine(Nap-dU)
gncacangnacnacnnganaggagcccgngccncagcc

SEQ ID NO: 112 - DNA, 37 bp, Artificial Sequence
  nucleic acid ligand AP048, wherein n is 5-(N-(1-naphthylmethyl)carboxamide)-2'-deoxyuridine(Nap-dU)
ncacangnacnacnnganaggagcccgngccncagcc

SEQ ID NO: 113 - DNA, 29 bp, Artificial Sequence
  nucleic acid ligand AP050, wherein n is 5-(N-(1-naphthylmethyl)carboxamide)-2'-deoxyuridine(Nap-dU)
acnacnnganaggagcccgngccncagcc

SEQ ID NO: 114 - DNA, 28 bp, Artificial Sequence
  nucleic acid ligand AP051, wherein n is 5-(N-(1-naphthylmethyl)carboxamide)-2'-deoxyuridine(Nap-dU)
cnacnnganaggagcccgngccncagcc

SEQ ID NO: 115 - DNA, 17 bp, Artificial Sequence
  nucleic acid ligand AP052, wherein n is 5-(N-(1-naphthylmethyl)carboxamide)-2'-deoxyuridine(Nap-dU)
gagcccgngccncagcc

SEQ ID NO: 116 - DNA, 16 bp, Artificial Sequence
  nucleic acid ligand AP053, wherein n is 5-(N-(1-naphthylmethyl)carboxamide)-2'-deoxyuridine(Nap-dU)
agcccgngccncagcc

SEQ ID NO: 117 - DNA, 47 bp, Artificial Sequence
  nucleic acid ligand AP054, wherein n is 5-(N-(1-naphthylmethyl)carboxamide)-2'-deoxyuridine(Nap-dU)
gccnggagcanggncacangnacnacnnganaggagcccgngccnca

SEQ ID NO: 118 - DNA, 46 bp, Artificial Sequence
  nucleic acid ligand AP055, wherein n is 5-(N-(1-naphthylmethyl)carboxamide)-2'-deoxyuridine(Nap-dU)
gccnggagcanggncacangnacnacnnganaggagcccgngccnc

SEQ ID NO: 119 - DNA, 74 bp, Artificial Sequence
  nucleic acid ligand AV001, wherein n is 5-(N-(1-naphthylmethyl)carboxamide)-2'-deoxyuridine(Nap-dU)
gagtgaccgtctgcctgagcaggaggangngacacaacnnngcannncaagccngancagccacaccaccagcc

SEQ ID NO: 120 - DNA, 60 bp, Artificial Sequence
  nucleic acid ligand AV002, wherein n is 5-(N-(1-naphthylmethyl)carboxamide)-2'-deoxyuridine(Nap-dU)
ctgagcaggaggangngacacaacnnngcannncaagccngancagccacaccaccagcc

SEQ ID NO: 121 - DNA, 46 bp, Artificial Sequence
  nucleic acid ligand AV003, wherein n is 5-(N-(1-naphthylmethyl)carboxamide)-2'-deoxyuridine(Nap-dU)
ctgagcaggaggangngacacaacnnngcannncaagccngancag

SEQ ID NO: 122 - DNA, 40 bp, Artificial Sequence
  nucleic acid ligand AV004, wherein n is 5-(N-(1-naphthylmethyl)carboxamide)-2'-deoxyuridine(Nap-dU)
agcaggaggangngacacaacnnngcannncaagccngan

SEQ ID NO: 123 - DNA, 33 bp, Artificial Sequence
  nucleic acid ligand AV005, wherein n is 5-(N-(1-naphthylmethyl)carboxamide)-2'-deoxyuridine(Nap-dU)
ccgtctgcctgagcaggaggangngacacaacn

SEQ ID NO: 124 - DNA, 74 bp, Artificial Sequence
  nucleic acid ligand AV006, wherein n is 5-(N-(1-naphthylmethyl)carboxamide)-2'-deoxyuridine(Nap-dU)
gagtgaccgtctgcctgngagaannangnaccnnaacgancanccgaaggnnnngaccagccacaccaccagcc

SEQ ID NO: 125 - DNA, 50 bp, Artificial Sequence
  nucleic acid ligand AV007, wherein n is 5-(N-(1-naphthylmethyl)carboxamide)-2'-deoxyuridine(Nap-dU)
gtctgcctgngagaannangnaccnnaacgancanccgaaggnnnngacc

SEQ ID NO: 126 - DNA, 42 bp, Artificial Sequence
  nucleic acid ligand AV008, wherein n is 5-(N-(1-naphthylmethyl)carboxamide)-2'-deoxyuridine(Nap-dU)
ngagaannangnaccnnaacgancanccgaaggnnnngacca

SEQ ID NO: 127 - DNA, 36 bp, Artificial Sequence
  nucleic acid ligand AV009, wherein n is 5-(N-(1-naphthylmethyl)carboxamide)-2'-deoxyuridine(Nap-dU)
annangnaccnnaacgancanccgaaggnnnngacc

SEQ ID NO: 128 - DNA, 74 bp, Artificial Sequence
  nucleic acid ligand IC001, wherein n is 5-(N-(1-naphthylmethyl)carboxamide)-2'-deoxyuridine(Nap-dU)
gagtgaccgtctgcctgaaagnccgganggcagcnnnacangcagaacnaacgnacacagccacaccaccagcc

SEQ ID NO: 129 - DNA, 57 bp, Artificial Sequence
  nucleic acid ligand IC002, wherein n is 5-(N-(1-naphthylmethyl)carboxamide)-2'-deoxyuridine(Nap-dU)
gagtgaccgtctgcctgaaagnccgganggcagcnnnacangcagaacnaacgnaca

SEQ ID NO: 130 - DNA, 44 bp, Artificial Sequence
  nucleic acid ligand IC003, wherein n is 5-(N-(1-naphthylmethyl)carboxamide)-2'-deoxyuridine(Nap-dU)
gagtgaccgtctgcctgaaagnccgganggcagcnnnacangca

SEQ ID NO: 131 - DNA, 40 bp, Artificial Sequence
  nucleic acid ligand IC004, wherein n is 5-(N-(1-naphthylmethyl)carboxamide)-2'-deoxyuridine(Nap-dU)
aaagnccgganggcagcnnnacangcagaacnaacgnaca

SEQ ID NO: 132 - DNA, 39 bp, Artificial Sequence
  nucleic acid ligand IC005, wherein n is 5-(N-(1-naphthylmethyl)carboxamide)-2'-deoxyuridine(Nap-dU)
accgtctgcctgaaagnccgganggcagcnnnacangca

SEQ ID NO: 133 - DNA, 34 bp, Artificial Sequence
  nucleic acid ligand IC006, wherein n is 5-(N-(1-naphthylmethyl)carboxamide)-2'-deoxyuridine(Nap-dU)
ctgcctgaaagnccgganggcagcnnnacangca

SEQ ID NO: 134 - DNA, 73 bp, Artificial Sequence
  nucleic acid ligand IC007, wherein n is 5-(N-(1-naphthylmethyl)carboxamide)-2'-deoxyuridine(Nap-dU)
gagtgaccgtctgcctggaccagcanaagnccgganggcagcnnnangccgaccancagccacaccaccagcc

SEQ ID NO: 135 - DNA, 49 bp, Artificial Sequence
  nucleic acid ligand IC008, wherein n is 5-(N-(1-naphthylmethyl)carboxamide)-2'-deoxyuridine(Nap-dU)
ctgcctggaccagcanaagnccgganggcagcnnnangccgaccancag

SEQ ID NO: 136 - DNA, 45 bp, Artificial Sequence
  nucleic acid ligand IC009, wherein n is 5-(N-(1-naphthylmethyl)carboxamide)-2'-deoxyuridine(Nap-dU)
ctgcctggaccagcanaagnccgganggcagcnnnangccgacca

SEQ ID NO: 137 - DNA, 40 bp, Artificial Sequence
  nucleic acid ligand IC010, wherein n is 5-(N-(1-naphthylmethyl)carboxamide)-2'-deoxyuridine(Nap-dU)
ctgcctggaccagcanaagnccgganggcagcnnnangcc

SEQ ID NO: 138 - DNA, 36 bp, Artificial Sequence
  nucleic acid ligand IC011, wherein n is 5-(N-(1-naphthylmethyl)carboxamide)-2'-deoxyuridine(Nap-dU)
ctggaccagcanaagnccgganggcagcnnnangcc

SEQ ID NO: 139 - DNA, 73 bp, Artificial Sequence
  nucleic acid ligand ID0001, wherein n is 5-(N-(1-naphthylmethyl)carboxamide)-2'-deoxyuridine(Nap-dU)
gagtgaccgtctgcctggacnagcanaagnccgganggcagcnnnangccgaccancagccacaccaccagcc

SEQ ID NO: 140 - DNA, 53 bp, Artificial Sequence
  nucleic acid ligand ID0002, wherein n is 5-(N-(1-naphthylmethyl)carboxamide)-2'-deoxyuridine(Nap-dU)
ctgcctggacnagcanaagnccgganggcagcnnnangccgaccancagccac

SEQ ID NO: 141 - DNA, 40 bp, Artificial Sequence
  nucleic acid ligand ID0003, wherein n is 5-(N-(1-naphthylmethyl)carboxamide)-2'-deoxyuridine(Nap-dU)
ctgcctggacnagcanaagnccgganggcagcnnnangcc

SEQ ID NO: 142 - DNA, 36 bp, Artificial Sequence
  nucleic acid ligand ID0004, wherein n is 5-(N-(1-naphthylmethyl)carboxamide)-2'-deoxyuridine(Nap-dU)
ctggacnagcanaagnccgganggcagcnnnangcc

SEQ ID NO: 143 - DNA, 59 bp, Artificial Sequence
  nucleic acid ligand ID0005, wherein n is 5-(N-(1-naphthylmethyl)carboxamide)-2'-deoxyuridine(Nap-dU)
ctggacnagcanaagnccgganggcagcnnnangccgaccancagccacaccaccagcc

SEQ ID NO: 144 - DNA, 73 bp, Artificial Sequence
  nucleic acid ligand TC001, wherein n is 5-(N-(1-naphthylmethyl)carboxamide)-2'-deoxyuridine(Nap-dU)
gagtgaccgtctgcctggacnagcataagnccgganggcagcnnnangccgaccancagccacaccaccagcc

SEQ ID NO: 145 - DNA, 53 bp, Artificial Sequence
  nucleic acid ligand TC002, wherein n is 5-(N-(1-naphthylmethyl)carboxamide)-2'-deoxyuridine(Nap-dU)
ctgcctggacnagcataagnccgganggcagcnnnangccgaccancagccac

SEQ ID NO: 146 - DNA, 42 bp, Artificial Sequence
  nucleic acid ligand TC003, wherein n is 5-(N-(1-naphthylmethyl)carboxamide)-2'-deoxyuridine(Nap-dU)
ctggacnagcataagnccgganggcagcnnnangccgaccan

SEQ ID NO: 147 - DNA, 40 bp, Artificial Sequence
  nucleic acid ligand TC004, wherein n is 5-(N-(1-naphthylmethyl)carboxamide)-2'-deoxyuridine(Nap-dU)
ctgcctggacnagcataagnccgganggcagcnnnangcc

SEQ ID NO: 148 - DNA, 36 bp, Artificial Sequence
  nucleic acid ligand TC005, wherein n is 5-(N-(1-naphthylmethyl)carboxamide)-2'-deoxyuridine(Nap-dU)
ctggacnagcataagnccgganggcagcnnnangcc

SEQ ID NO: 149 - DNA, 74 bp, Artificial Sequence
  nucleic acid ligand TD001, wherein n is 5-(N-(1-naphthylmethyl)carboxamide)-2'-deoxyuridine(Nap-dU)
gagtgaccgtctgcctgggacnagcanaagnccgganggcagcnnnangccgaccancagccacaccaccagcc

SEQ ID NO: 150 - DNA, 47 bp, Artificial Sequence
  nucleic acid ligand TD002, wherein n is 5-(N-(1-naphthylmethyl)carboxamide)-2'-deoxyuridine(Nap-dU)
ctgcctgggacnagcanaagnccgganggcagcnnnangccgaccan

SEQ ID NO: 151 - DNA, 40 bp, Artificial Sequence
  nucleic acid ligand TD003, wherein n is 5-(N-(1-naphthylmethyl)carboxamide)-2'-deoxyuridine(Nap-dU)
ggacnagcanaagnccgganggcagcnnnangccgaccan

SEQ ID NO: 152 - DNA, 32 bp, Artificial Sequence
  nucleic acid ligand TD004, wherein n is 5-(N-(1-naphthylmethyl)carboxamide)-2'-deoxyuridine(Nap-dU)
ctgcctgggacnagcanaagnccgganggcag

SEQ ID NO: 153 - DNA, 74 bp, Artificial Sequence
  nucleic acid ligand TD005, wherein n is 5-(N-(1-naphthylmethyl)carboxamide)-2'-deoxyuridine(Nap-dU)
gagtgaccgtctgcctgaaagnccgganggcagcnnnacaggcagaacnaacgnacacagccacaccaccagcc

SEQ ID NO: 154 - DNA, 53 bp, Artificial Sequence
  nucleic acid ligand TD006, wherein n is 5-(N-(1-naphthylmethyl)carboxamide)-2'-deoxyuridine(Nap-dU)
gagtgaccgtctgcctgaaagnccgganggcagcnnnacaggcagaacnaacg

SEQ ID NO: 155 - DNA, 48 bp, Artificial Sequence
  nucleic acid ligand TD007, wherein n is 5-(N-(1-naphthylmethyl)carboxamide)-2'-deoxyuridine(Nap-dU)
accgtctgcctgaaagnccgganggcagcnnnacaggcagaacnaacg

SEQ ID NO: 156 - DNA, 35 bp, Artificial Sequence
  nucleic acid ligand TD008, wherein n is 5-(N-(1-naphthylmethyl)carboxamide)-2'-deoxyuridine(Nap-dU)
ctgcctgaaagnccgganggcagcnnnacaggcag

SEQ ID NO: 157 - DNA, 74 bp, Artificial Sequence
  nucleic acid ligand TD009, wherein n is 5-(N-(1-naphthylmethyl)carboxamide)-2'-deoxyuridine(Nap-dU)
gagtgaccgtctgcctgganangccncnncngcagnnacggngngancgcccaanagcagccacaccaccagcc

SEQ ID NO: 158 - DNA, 57 bp, Artificial Sequence
  nucleic acid ligand TD010, wherein n is 5-(N-(1-naphthylmethyl)carboxamide)-2'-deoxyuridine(Nap-dU)
ctgcctgganangccncnncngcagnnacggngngancgcccaanagcagccacacc

SEQ ID NO: 159 - DNA, 47 bp, Artificial Sequence
  nucleic acid ligand TD011, wherein n is 5-(N-(1-naphthylmethyl)carboxamide)-2'-deoxyuridine(Nap-dU)
angccncnncngcagnnacggngngancgcccaanagcagccacacc

SEQ ID NO: 160 - DNA, 44 bp, Artificial Sequence
  nucleic acid ligand TD012, wherein n is 5-(N-(1-naphthylmethyl)carboxamide)-2'-deoxyuridine(Nap-dU)
angccncnncngcagnnacggngngancgcccaanagcagccac

SEQ ID NO: 161 - DNA, 34 bp, Artificial Sequence
  nucleic acid ligand TD013, wherein n is 5-(N-(1-naphthylmethyl)carboxamide)-2'-deoxyuridine(Nap-dU)
caggncgagcngnacgcgngngngaccngaagac

SEQ ID NO: 162 - DNA, 34 bp, Artificial Sequence; identical to SEQ ID NO: 161
  nucleic acid ligand AD043, wherein n is 5-(N-(1-naphthylmethyl)carboxamide)-2'-deoxyuridine(Nap-dU)

SEQ ID NO: 163 - DNA, 39 bp, Artificial Sequence
  nucleic acid ligand AD044, wherein n is 5-(N-(1-naphthylmethyl)carboxamide)-2'-deoxyuridine(Nap-dU)
caggncgagcngnacgcgngngngaccngaagacgnana

SEQ ID NO: 164 - DNA, 44 bp, Artificial Sequence
  nucleic acid ligand AD045, wherein n is 5-(N-(1-naphthylmethyl)carboxamide)-2'-deoxyuridine(Nap-dU)
caggncgagcngnacgcgngngngaccngaagacgnanaacnnn

SEQ ID NO: 165 - DNA, 49 bp, Artificial Sequence
  nucleic acid ligand AD046, wherein n is 5-(N-(1-naphthylmethyl)carboxamide)-2'-deoxyuridine(Nap-dU)
caggncgagcngnacgcgngngngaccngaagacgnanaacnnnnacag

SEQ ID NO: 166 - DNA, 54 bp, Artificial Sequence
  nucleic acid ligand AD047, wherein n is 5-(N-(1-naphthylmethyl)carboxamide)-2'-deoxyuridine(Nap-dU)
caggncgagcngnacgcgngngngaccngaagacgnanaacnnnnacagaancn

SEQ ID NO: 167 - DNA, 28 bp, Artificial Sequence
  nucleic acid ligand AD048, wherein n is 5-(N-(1-naphthylmethyl)carboxamide)-2'-deoxyuridine(Nap-dU)
aagacgnanaacnnnnacagaancnaca

SEQ ID NO: 168 - DNA, 33 bp, Artificial Sequence
  nucleic acid ligand AD049, wherein n is 5-(N-(1-naphthylmethyl)carboxamide)-2'-deoxyuridine(Nap-dU)
accngaagacgnanaacnnnnacagaancnaca

SEQ ID NO: 169 - DNA, 38 bp, Artificial Sequence
  nucleic acid ligand AD050, wherein n is 5-(N-(1-naphthylmethyl)carboxamide)-2'-deoxyuridine(Nap-dU)
gngngaccngaagacgnanaacnnnnacagaancnaca

SEQ ID NO: 170 - DNA, 43 bp, Artificial Sequence
  nucleic acid ligand AD051, wherein n is 5-(N-(1-naphthylmethyl)carboxamide)-2'-deoxyuridine(Nap-dU)
cgcgngngngaccngaagacgnanaacnnnnacagaancnaca

SEQ ID NO: 171 - DNA, 48 bp, Artificial Sequence
  nucleic acid ligand AD052, wherein n is 5-(N-(1-naphthylmethyl)carboxamide)-2'-deoxyuridine(Nap-dU)
cngnacgcgngngngaccngaagacgnanaacnnnnacagaancnaca

SEQ ID NO: 172 - DNA, 53 bp, Artificial Sequence
  nucleic acid ligand AD053, wherein n is 5-(N-(1-naphthylmethyl)carboxamide)-2'-deoxyuridine(Nap-dU)
ncgagcngnacgcgngngngaccngaagacgnanaacnnnnacagaancnaca

SEQ ID NO: 173 - DNA, 74 bp, Artificial Sequence
  nucleic acid ligand AX001, wherein n is 5-(N-(1-naphthylmethyl)carboxamide)-2'-deoxyuridine(Nap-dU)
gagtgaccgtctgcctgnacganaacngagngnangcannagaccnnnngngaccgncagccacaccaccagcc

SEQ ID NO: 174 - DNA, 52 bp, Artificial Sequence
  nucleic acid ligand AX002, wherein n is 5-(N-(1-naphthylmethyl)carboxamide)-2'-deoxyuridine(Nap-dU)
cgtctgcctgnacganaacngagngnatngcannagaccnnnngngaccgnc

SEQ ID NO: 175 - DNA, 42 bp, Artificial Sequence
  nucleic acid ligand AX003, wherein n is 5-(N-(1-naphthylmethyl)carboxamide)-2'-deoxyuridine(Nap-dU)
gagngnangcannagaccnnnngngaccgncagccacaccac

SEQ ID NO: 176 - DNA, 35 bp, Artificial Sequence
  nucleic acid ligand AX004, wherein n is 5-(N-(1-naphthylmethyl)carboxamide)-2'-deoxyuridine(Nap-dU)
annagaccnnnngngaccgncagccacaccaccag

SEQ ID NO: 177 - DNA, 30 bp, Artificial Sequence
  nucleic acid ligand AX005, wherein n is 5-(N-(1-naphthylmethyl)carboxamide)-2'-deoxyuridine(Nap-dU)
anaacngagngnangcannagaccnnnngn

SEQ ID NO: 178 - DNA, 79 bp, Artificial Sequence
  nucleic acid ligand IV001, wherein n is 5-(N-(1-naphthylmethyl)carboxamide)-2'-deoxyuridine(Nap-dU)
gagtgaccgtctgcctgngngagaannangnacccnnaacgancanccgaaggnnnngaccacagccacaccaccagcc

SEQ ID NO: 179 - DNA, 65 bp, Artificial Sequence
  nucleic acid ligand IV002, wherein n is 5-(N-(1-naphthylmethyl)carboxamide)-2'-deoxyuridine(Nap-dU)
ctgngngagaannangnacccnnaacgancanccgaaggnnnngaccacagccacaccaccagcc

SEQ ID NO: 180 - DNA, 50 bp, Artificial Sequence
  nucleic acid ligand IV003, wherein n is 5-(N-(1-naphthylmethyl)carboxamide)-2'-deoxyuridine(Nap-dU)
gnacccnnaacgancanccgaaggnnnngaccacagccacaccaccagcc

SEQ ID NO: 181 - DNA, 44 bp, Artificial Sequence
  nucleic acid ligand IV004, wherein n is 5-(N-(1-naphthylmethyl)carboxamide)-2'-deoxyuridine(Nap-dU)
nnaacgancanccgaaggnnnngaccacagccacaccaccagcc

SEQ ID NO: 182 - DNA, 39 bp, Artificial Sequence
  nucleic acid ligand IV005, wherein n is 5-(N-(1-naphthylmethyl)carboxamide)-2'-deoxyuridine(Nap-dU)
nnaacgancanccgaaggnnnngaccacagccacaccac

SEQ ID NO: 183 - DNA, 45 bp, Artificial Sequence
  nucleic acid ligand IV006, wherein n is 5-(N-(1-naphthylmethyl)carboxamide)-2'-deoxyuridine(Nap-dU)
ngngagaannangnacccnnaacgancanccgaaggnnnngacca

SEQ ID NO: 184 - DNA, 35 bp, Artificial Sequence
  aptamer KD003, wherein n is 5-(N-benzylcarboxamide)-2'-deoxyuridine(Bz-dU)
accngnngcagcaccnanncanacggacgcncncn

SEQ ID NO: 185 - DNA, 40 bp, Artificial Sequence
  aptamer KD006, wherein n is 5-(N-benzylcarboxamide)-2'-deoxyuridine(Bz-dU)
gngncaccngnngcagcaccnanncanacggacgcncncn